European Patent Application EP 4 484 417 A1, published January 1, 2025. Title: NOVEL POMALIDOMIDE DERIVATIVE, PREPARATION METHOD THEREFOR, AND USE THEREOF. Applicant: Aevis Bio, Inc. The sequence listing filed with the application follows.

SEQUENCE LISTING (22 sequences)

SEQ ID NO: 1 - DNA, 21 bp, synthetic construct
  source 1..21: mol_type = other DNA
cccagggacctctctctaatc

SEQ ID NO: 2 - DNA, 21 bp, synthetic construct
  source 1..21: mol_type = other DNA
atgggctacaggcttgtcact

SEQ ID NO: 3 - DNA, 21 bp, synthetic construct
  source 1..21: mol_type = other DNA
acagatgaagtgctccttcca

SEQ ID NO: 4 - DNA, 21 bp, synthetic construct
  source 1..21: mol_type = other DNA
gtcggagattcgtagctggat

SEQ ID NO: 5 - DNA, 20 bp, synthetic construct
  source 1..20: mol_type = other DNA
ggcactggcagaaaacaacc

SEQ ID NO: 6 - DNA, 21 bp, synthetic construct
  source 1..21: mol_type = other DNA
gcaagtctcctcattgaatcc

SEQ ID NO: 7 - DNA, 20 bp, synthetic construct
  source 1..20: mol_type = other DNA
agagtgattgagagtggacc

SEQ ID NO: 8 - DNA, 19 bp, synthetic construct
  source 1..19: mol_type = other DNA
acttctccacaaccctctg

SEQ ID NO: 9 - DNA, 21 bp, synthetic construct
  source 1..21: mol_type = other DNA
ggatgcagaaggagatcactg

SEQ ID NO: 10 - DNA, 20 bp, synthetic construct
  source 1..20: mol_type = other DNA
cgatccacacggagtacttg

SEQ ID NO: 11 - DNA, 20 bp, synthetic construct
  source 1..20: mol_type = other DNA
tagctcccagaaaagcaagc

SEQ ID NO: 12 - DNA, 20 bp, synthetic construct
  source 1..20: mol_type = other DNA
ttttctggagggagatgtgg

SEQ ID NO: 13 - DNA, 20 bp, synthetic construct
  source 1..20: mol_type = other DNA
ccggagaggagacttcacag

SEQ ID NO: 14 - DNA, 20 bp, synthetic construct
  source 1..20: mol_type = other DNA
cagaattgccattgcacaac

SEQ ID NO: 15 - DNA, 20 bp, synthetic construct
  source 1..20: mol_type = other DNA
gaagaagtgcccatcctctg

SEQ ID NO: 16 - DNA, 20 bp, synthetic construct
  source 1..20: mol_type = other DNA
agctcatatgggtccgacag

SEQ ID NO: 17 - DNA, 24 bp, synthetic construct
  source 1..24: mol_type = other DNA
ttcaacagcaactcccactcttcc

SEQ ID NO: 18 - DNA, 23 bp, synthetic construct
  source 1..23: mol_type = other DNA
tggtccagggtttcttactcctt

SEQ ID NO: 19 - DNA, 20 bp, synthetic construct
  source 1..20: mol_type = other DNA
gctatggccgctttgatgtg

SEQ ID NO: 20 - DNA, 20 bp, synthetic construct
  source 1..20: mol_type = other DNA
ttgggatgctccatggtcac

SEQ ID NO: 21 - DNA, 25 bp, synthetic construct
  source 1..25: mol_type = other DNA
ctggaacatggactcactcagtttg

SEQ ID NO: 22 - DNA, 20 bp, synthetic construct
  source 1..20: mol_type = other DNA
aggcctttgccactgcttgt